European Patent Application EP 4 800 113 A1, published September 2, 2026. Title: Microorganism having enhanced activity of phosphotransacetylase-acetate kinase operon and uses thereof. Applicant: CJ CheilJedang Corporation. The sequence listing filed with the application follows.

SEQUENCE LISTING (33 sequences)

SEQ ID NO: 1 - protein, 461 aa, synthetic construct
  REGION 1..461: note = Pta (phosphotransacetylase) (Sequence ID: WP_003862872.1)
MSDTPTSALITTVNRSFDGFDLEEVAADLGVRLTNLPDEELEVSKVLAADLLAEGPALIIGVGNTFFDAQVAAALGVPVLLLVDKQGKHVALARTQVNNAGAVVAAAFTAEQEPMPDKLRKAVRNHSNLEPVMSAELFENWLLKRARAEHSHIVLPEGDDDRILMAAHQLLDQDICDITILGDPVKIKERATELGLHLNTAYLVNPLTDPRLEEFAEQFAELRKSKSVTIDEAREIMKDISYFGTMMVHNGDADGMVSGAANTTAHTIKPSFQIIKTVPEASVVSSIFLMVLRGRLWAFGDCAVNPNPTAEQLGEIAVVSAKTAAQFGIDPRVAILSYSTGNSGGGSDVDRAIDALAEARRLNPELCVDGPLQFDAAVDPGVARKKMPDSDVAGQANVFIFPDLEAGNIGYKTAQRTGHALAVGPILQGLNKPVNDLSRGATVPDIVNTVAITAIQAGGRS

SEQ ID NO: 2 - DNA, 1386 bp, synthetic construct
  misc_feature 1..1386: note = gene coding Pta
  source 1..1386: mol_type = other DNA
atgtctgacacaccgacctcagctctgatcaccacggtcaaccgcagcttcgatggattcgatttggaagaagtagcagcagaccttggagttcggctcaccaacctgcccgacgaagaactagaagtatccaaagttctcgcggcggacctcctcgctgaggggccagctctcatcatcggtgtaggaaacacgtttttcgacgcccaggtcgccgctgccctcggcgtcccagtgctactgctggtagacaagcaaggcaagcacgttgctcttgctcgcacccaggtaaacaatgccggcgcagttgttgcagcagcatttaccgctgaacaagagccaatgccggataagctgcgcaaggctgtgcgcaaccacagcaacctcgaaccagtcatgagcgccgaactctttgaaaactggctgctcaagcgcgcacgcgcagagcactcccacattgtgctgccagaaggtgacgacgaccgcatcttgatggctgcccaccagctgcttgaccaagacatctgtgacatcacgatccttggcgatccagtaaagatcaaggagcgcgctaccgaacttggcctgcaccttaacactgcatacctggtcaatccgctgacagatcctcgcctggaggaattcgccgaacaattcgcggagctgcgcaagtcaaagagcgtcactatcgatgaagcccgcgaaatcatgaaggatatttcctacttcggcaccatgatggtccacaacggcgacgccgacggaatggtatccggtgcagcaaacaccaccgcacacaccattaagccaagcttccagatcatcaaaactgttccagaagcatccgtcgtttcttccatcttcctcatggtgctgcgcgggcgactgtgggcattcggcgactgtgctgttaacccgaacccaactgctgaacagcttggtgaaatcgccgttgtgtcagcaaaaactgcagcacaatttggcattgatcctcgcgtagccatcttgtcctactccactggcaactccggcggaggctcagatgtggatcgcgccatcgacgctcttgcagaagcacgccgactcaacccagaactatgcgtcgatggaccacttcagttcgacgccgccgtcgacccgggtgtggcgcgcaagaagatgccagactctgacgtcgctggccaggcaaatgtgtttatcttccctgacctggaagccggaaacatcggctacaaaactgcacaacgcaccggtcacgccctggcagttggtccgattctgcagggcctgaacaaaccagtcaacgacctttcccgtggcgcaacagtccctgacatcgtcaacacagtagccatcaccgcaattcaggcaggaggacgcagctaa

SEQ ID NO: 3 - protein, 397 aa, synthetic construct
  REGION 1..397: note = ackA (acetate kinase) (Sequence ID: WP_003862874.1)
MALALVLNSGSSSIKFQLVNPENSAIDEPYVSGLVEQIGEPNGRIVLKIEGEKYTLETPIADHSEGLNLAFDLMDQHNCGPSQLEITAVGHRVVHGGILFSAPELITDEIVEMIRDLIPLAPLHNPANVDGIDVARKILPDVPHVAVFDTGFFHSLPPAAALYAINKDVAAEHGIRRYGFHGTSHEFVSKRVVEILEKPTEDINTITFHLGNGASMAAVQGGRAVDTSMGMTPLAGLVMGTRSGDIDPGIVFHLSRTAGMSIDEIDNLLNKKSGVKGLSGVNDFRELREMIDNNDQDAWSAYNIYIHQLRRYLGSYMVALGRVDTIVFTAGVGENAQFVREDALAGLEMYGIEIDPERNALPNDGPRLISTDASKVKVFVIPTNEELAIARYAVKFA

SEQ ID NO: 4 - DNA, 1194 bp, synthetic construct
  misc_feature 1..1194: note = gene coding ackA
  source 1..1194: mol_type = other DNA
atggcattggcacttgttttgaactccggttcatcttccatcaaattccagctggtcaaccccgaaaactctgccatcgacgagccatatgtttctggtcttgtggagcagattggtgagccaaacggccgcatcgtactcaaaatagagggtgaaaaatacaccctagagacacccatcgcagatcactccgaaggcctaaacctggcgttcgatctcatggaccagcacaactgtggtccttcccaactggaaatcaccgcagttggacaccgcgtggtccacggtggaatcttgttctctgcaccggaacttatcactgatgaaatcgttgaaatgatccgcgatctcattccactcgcaccactgcacaaccctgcaaacgttgacggcattgatgttgctcgaaaaattctccccgatgtcccacacgtagctgtctttgacaccggtttcttccactcacttccaccagcagctgcgctgtatgccatcaataaagatgttgccgctgaacacggaatcaggcgctatggtttccacggcacctctcatgaatttgtgtccaagcgcgtggtggaaattctggaaaagcccaccgaagacatcaacaccatcaccttccacctgggcaacggcgcatccatggctgctgttcaaggcggccgtgcggtagatacttccatgggtatgacacctctcgcgggacttgtcatgggtacccgaagcggtgacattgatccaggtatcgttttccatctctcacgcaccgctggcatgagcatcgatgagatcgataacctactgaacaagaagtcgggcgttaaaggtctttccggagtcaatgatttccgtgaactgcgggaaatgatcgacaacaatgatcaagatgcctggtccgcgtacaacatttacatacaccaactccgccgctacctcggttcctacatggtggcactgggacgggtagacaccatcgtgttcaccgccggtgtcggtgaaaatgcccagtttgtccgtgaggatgccttggcaggtttggaaatgtacggcatcgaaatcgatccggagcgcaacgcactgccaaacgatggtcctcgattgatttccactgatgcctccaaggtgaaggtgtttgtcatcccaactaatgaagaattagctatcgctaggtacgcggtgaagttcgcttag

SEQ ID NO: 5 - DNA, 369 bp, synthetic construct
  misc_feature 1..369: note = ctaE promoter (PctaE)
  source 1..369: mol_type = other DNA
catgaatcgcattaagctgcaaaaacgccttttattcgggttcaaccaaaagttgtatgtggggctccaatggggtgaaaaactctgtgacgtgtctctcaggcaaaaacctgcggaaaccactttgggcacactctgtgagttcttcaaaatgggacgagtgtgatttgggacagattggaactgcctgtgaaccctttaacctgcaattatgtaactgtcgtaaaagggctatgaagagttcccggaaggtcgattgaaaagtttgcgaattgggggaaaattcgcatcaaaagccgagttcaaactttcaattgaaacggggggcttgaagtgactttggccaaccaaacagccatactagatagc

SEQ ID NO: 6 - DNA, 490 bp, synthetic construct
  misc_feature 1..490: note = pyk promoter (Ppyk)
  source 1..490: mol_type = other DNA
ctctacgtagctggttacaccttgggccgtttctggattgaacaaatgcgcgttgatgaagccacgcttattggcggcatccgaatcaacaccatcgtctccgcagtagtgtttgccggcgcgatcattgtgttcttcctgttgaagaagggtagggaaactcccgaagaggtagatccgactttcacagcgtctgttgcagcagatgctgtagcttcgccagatggaaaacccttgccgaaagcagaggagggcattgatggagaaacgccctcaacgcgataggtttcaaccataggcctgacctggctgagatgtttttggtagaaaaaccgagtgcccgaattgttttgtgggtgcccggtttttctgatttaagcacgtcagaggcgtagaacattgtctgttcacactctgggtcgcaagattcatcgagaattaatggtagtatctgtggcttgagggggaatgacgtactaggcttatgggc

SEQ ID NO: 7 - DNA, 500 bp, synthetic construct
  misc_feature 1..500: note = pfkA promoter (PpfkA)
  source 1..500: mol_type = other DNA
ttcttggcaagtgggtgggacaggccaaatgcaccaacgtaggttgccagcaggccagtagctactgcaggacccttcttttcattccagcttcgtgcagcaagcgctccggatgctgccaatggaatggtgcccagtgggcgaatgccggattcacgggcagtcaaccaaccgccgatcaaacctgctgcgacgacggtggcagtgctgacctgggatgcctttttcaatttcatttccatggtgagccagtctagagacaaaatttttccgcgggggttttcttgatctgatccgacaacccaatgggggcaaaaatgtgtccgaccaaaaattgtgcagcacaccacatgcccgctcggacaatgtcgatttgttaatgaaactgcagctctggcgattaaataagatggtcagagacagttttttggcctgtcaacccctgtgattctcttatttttgggtgattgttccggcgcgggtgttgtgatgggtttaat

SEQ ID NO: 8 - DNA, 40 bp, synthetic construct
  misc_feature 1..40: note = primer
  source 1..40: mol_type = other DNA
gctcggtacccggggatcccgtccgtgtcggatttcatca

SEQ ID NO: 9 - DNA, 29 bp, synthetic construct
  misc_feature 1..29: note = primer
  source 1..29: mol_type = other DNA
ctcgagacatcgcctttctagtttcagcc

SEQ ID NO: 10 - DNA, 24 bp, synthetic construct
  misc_feature 1..24: note = primer
  source 1..24: mol_type = other DNA
atgtctgacacaccgacctcagct

SEQ ID NO: 11 - DNA, 40 bp, synthetic construct
  misc_feature 1..40: note = primer
  source 1..40: mol_type = other DNA
cctgcaggtcgactctagaagtgttaaggtgcaggccaag

SEQ ID NO: 12 - DNA, 43 bp, synthetic construct
  misc_feature 1..43: note = primer
  source 1..43: mol_type = other DNA
aaaggcgatgtctcgagcatgaatcgcattaagctgcaaaaac

SEQ ID NO: 13 - DNA, 41 bp, synthetic construct
  misc_feature 1..41: note = primer
  source 1..41: mol_type = other DNA
tcggtgtgtcagacatgctatctagtatggctgtttggttg

SEQ ID NO: 14 - DNA, 40 bp, synthetic construct
  misc_feature 1..40: note = primer
  source 1..40: mol_type = other DNA
aaaggcgatgtctcgagctctacgtagctggttacacctt

SEQ ID NO: 15 - DNA, 38 bp, synthetic construct
  misc_feature 1..38: note = primer
  source 1..38: mol_type = other DNA
tcggtgtgtcagacatgcccataagcctagtacgtcat

SEQ ID NO: 16 - DNA, 37 bp, synthetic construct
  misc_feature 1..37: note = primer
  source 1..37: mol_type = other DNA
aaaggcgatgtctcgagttcttggcaagtgggtggga

SEQ ID NO: 17 - DNA, 39 bp, synthetic construct
  misc_feature 1..39: note = primer
  source 1..39: mol_type = other DNA
tcggtgtgtcagacatattaaacccatcacaacacccgc

SEQ ID NO: 18 - DNA, 41 bp, synthetic construct
  misc_feature 1..41: note = primer
  source 1..41: mol_type = other DNA
gctcggtacccggggatcccgatccatgctggtagaaatca

SEQ ID NO: 19 - DNA, 25 bp, synthetic construct
  misc_feature 1..25: note = primer
  source 1..25: mol_type = other DNA
gttcaagtttgctgccatcccaggt

SEQ ID NO: 20 - DNA, 26 bp, synthetic construct
  misc_feature 1..26: note = primer
  source 1..26: mol_type = other DNA
ttggctcaaattagtgccgaaggcga

SEQ ID NO: 21 - DNA, 40 bp, synthetic construct
  misc_feature 1..40: note = primer
  source 1..40: mol_type = other DNA
cctgcaggtcgactctagacatgcaatggtagacgctcag

SEQ ID NO: 22 - DNA, 44 bp, synthetic construct
  misc_feature 1..44: note = primer
  source 1..44: mol_type = other DNA
tggcagcaaacttgaactccttaaaggggttttaaaaaatgtgg

SEQ ID NO: 23 - DNA, 41 bp, synthetic construct
  misc_feature 1..41: note = primer
  source 1..41: mol_type = other DNA
tcggcactaatttgagccaactaagcgaacttcaccgcgta

SEQ ID NO: 24 - DNA, 42 bp, synthetic construct
  misc_feature 1..42: note = primer
  source 1..42: mol_type = other DNA
tggcagcaaacttgaaccatgaatcgcattaagctgcaaaaa

SEQ ID NO: 25 - DNA, 42 bp, synthetic construct
  misc_feature 1..42: note = primer
  source 1..42: mol_type = other DNA
aggtcggtgtgtcagacatgctatctagtatggctgtttggt

SEQ ID NO: 26 - DNA, 24 bp, synthetic construct
  misc_feature 1..24: note = primer
  source 1..24: mol_type = other DNA
atgtctgacacaccgacctcagct

SEQ ID NO: 27 - DNA, 41 bp, synthetic construct
  misc_feature 1..41: note = primer
  source 1..41: mol_type = other DNA
cggggatcccccgggaggacggtactcaaatactaaacttc

SEQ ID NO: 28 - DNA, 38 bp, synthetic construct
  misc_feature 1..38: note = primer
  source 1..38: mol_type = other DNA
tgccgagtgtttcggtctttacagacacgagggacacg

SEQ ID NO: 29 - DNA, 31 bp, synthetic construct
  misc_feature 1..31: note = primer
  source 1..31: mol_type = other DNA
tgtctgtaaagaccgaaacactcggcatcaa

SEQ ID NO: 30 - DNA, 41 bp, synthetic construct
  misc_feature 1..41: note = primer
  source 1..41: mol_type = other DNA
cggggatcccccggggacaactacattattattataccaca

SEQ ID NO: 31 - DNA, 2579 bp, synthetic construct
  misc_feature 1..2579: note = structural gene of pta-ackA operon
  source 1..2579: mol_type = other DNA
atgtctgacacaccgacctcagctctgatcaccacggtcaaccgcagcttcgatggattcgatttggaagaagtagcagcagaccttggagttcggctcaccaacctgcccgacgaagaactagaagtatccaaagttctcgcggcggacctcctcgctgaggggccagctctcatcatcggtgtaggaaacacgtttttcgacgcccaggtcgccgctgccctcggcgtcccagtgctactgctggtagacaagcaaggcaagcacgttgctcttgctcgcacccaggtaaacaatgccggcgcagttgttgcagcagcatttaccgctgaacaagagccaatgccggataagctgcgcaaggctgtgcgcaaccacagcaacctcgaaccagtcatgagcgccgaactctttgaaaactggctgctcaagcgcgcacgcgcagagcactcccacattgtgctgccagaaggtgacgacgaccgcatcttgatggctgcccaccagctgcttgaccaagacatctgtgacatcacgatccttggcgatccagtaaagatcaaggagcgcgctaccgaacttggcctgcaccttaacactgcatacctggtcaatccgctgacagatcctcgcctggaggaattcgccgaacaattcgcggagctgcgcaagtcaaagagcgtcactatcgatgaagcccgcgaaatcatgaaggatatttcctacttcggcaccatgatggtccacaacggcgacgccgacggaatggtatccggtgcagcaaacaccaccgcacacaccattaagccaagcttccagatcatcaaaactgttccagaagcatccgtcgtttcttccatcttcctcatggtgctgcgcgggcgactgtgggcattcggcgactgtgctgttaacccgaacccaactgctgaacagcttggtgaaatcgccgttgtgtcagcaaaaactgcagcacaatttggcattgatcctcgcgtagccatcttgtcctactccactggcaactccggcggaggctcagatgtggatcgcgccatcgacgctcttgcagaagcacgccgactcaacccagaactatgcgtcgatggaccacttcagttcgacgccgccgtcgacccgggtgtggcgcgcaagaagatgccagactctgacgtcgctggccaggcaaatgtgtttatcttccctgacctggaagccggaaacatcggctacaaaactgcacaacgcaccggtcacgccctggcagttggtccgattctgcagggcctgaacaaaccagtcaacgacctttcccgtggcgcaacagtccctgacatcgtcaacacagtagccatcaccgcaattcaggcaggaggacgcagctaatggcattggcacttgttttgaactccggttcatcttccatcaaattccagctggtcaaccccgaaaactctgccatcgacgagccatatgtttctggtcttgtggagcagattggtgagccaaacggccgcatcgtactcaaaatagagggtgaaaaatacaccctagagacacccatcgcagatcactccgaaggcctaaacctggcgttcgatctcatggaccagcacaactgtggtccttcccaactggaaatcaccgcagttggacaccgcgtggtccacggtggaatcttgttctctgcaccggaacttatcactgatgaaatcgttgaaatgatccgcgatctcattccactcgcaccactgcacaaccctgcaaacgttgacggcattgatgttgctcgaaaaattctccccgatgtcccacacgtagctgtctttgacaccggtttcttccactcacttccaccagcagctgcgctgtatgccatcaataaagatgttgccgctgaacacggaatcaggcgctatggtttccacggcacctctcatgaatttgtgtccaagcgcgtggtggaaattctggaaaagcccaccgaagacatcaacaccatcaccttccacctgggcaacggcgcatccatggctgctgttcaaggcggccgtgcggtagatacttccatgggtatgacacctctcgcgggacttgtcatgggtacccgaagcggtgacattgatccaggtatcgttttccatctctcacgcaccgctggcatgagcatcgatgagatcgataacctactgaacaagaagtcgggcgttaaaggtctttccggagtcaatgatttccgtgaactgcgggaaatgatcgacaacaatgatcaagatgcctggtccgcgtacaacatttacatacaccaactccgccgctacctcggttcctacatggtggcactgggacgggtagacaccatcgtgttcaccgccggtgtcggtgaaaatgcccagtttgtccgtgaggatgccttggcaggtttggaaatgtacggcatcgaaatcgatccggagcgcaacgcactgccaaacgatggtcctcgattgatttccactgatgcctccaaggtgaaggtgtttgtcatcccaactaatgaagaattagctatcgctaggtacgcggtgaagttcgcttag

SEQ ID NO: 32 - DNA, 502 bp, synthetic construct
  misc_feature 1..502: note = ald promoter (Pald)
  source 1..502: mol_type = other DNA
cgatcatcgaactcggcgaagaaaaccgaaacctcaaagaatccctgcgtaaggtcacagctgagaatgagcagctcaaagatcaattacgcagcgggcgtccgcgtggcgagctggtgcacgtgccccgctccaccgcggtggtcatgtgggaacgccgcaaggggcgttccaagtaaaaacatgcttgtcgacgccactttctagcaaattaagcgggcacctccatttatcttttggaggtgcccgtttcgtgctttcgccaattagatacatggataaccacccgaacagggggtaataacttttgaaaggctttcggcgttgagctgcgagaattttgagaaaaagggggtgaatttaacaggggttctagcgcggattgattttcgtgaatatggtggctgctaagcgtgcgaatgtgcgcgttatcacaatcgttgaccaagtgtcacctgacgcacaggtagtgctcaggtggaggtggcccaaaggagaccca

SEQ ID NO: 33 - DNA, 5802 bp, synthetic construct
  misc_feature 1..5802: note = pDC24 vector
  source 1..5802: mol_type = other DNA
gttcgcttgctgtccataaaaccgcccagtctagctatcgccatgtaagcccactgcaagctacctgctttctctttgcgcttgcgttttcccttgtccagatagcccagtagctgacattcatccggggtcagcaccgtttctgcggactggctttctacgtgttccgcttcctttagcagcccttgcgccctgagtgcttgcggcagcgtgaagctagcttttatcgccattcgccattcaggctgcgcaactgttgggaagggcgatcggtgcgggcctcttcgctattacgccagctggcgaaagggggatgtgctgcaaggcgattaagttgggtaacgccagggttttcccagtcacgacgttgtaaaacgacggccagtgaattcgagctcggtacccggggatcctctagagtcgacctgcaggcatgcaagcttggcgtaatcatggtcatagctgtttcctgtgtgaaattgttatccgctcacaattccacacaacatacgagccggaagcataaagtgtaaagcctggggtgcctaatgagtgagctaactcacattaattgcgttgcgctcactgcccgctttccagtcgggaaacctgtcgtgccagctgcattaatgaatcggccaacgcgcggggagaggcggtttgcgtattgggcgctcttccgcttcctcgctcactgactcgctgcgctcggtcgttcggctgcggcgagcggtatcagctcactcaaaggcggtaatacggttatccacagaatcaggggataacgcaggaaagaacatgtgagcaaaaggccagcaaaaggccaggaaccgtaaaaaggccgcgttgctggcgtttttccataggctccgcccccctgacgagcatcacaaaaatcgacgctcaagtcagaggtggcgaaacccgacaggactataaagataccaggcgtttccccctggaagctccctcgtgcgctctcctgttccgaccctgccgcttaccggatacctgtccgcctttctcccttcgggaagcgtggcgctttctcaatgctcacgctgtaggtatctcagttcggtgtaggtcgttcgctccaagctgggctgtgtgcacgaaccccccgttcagcccgaccgctgcgccttatccggtaactatcgtcttgagtccaacccggtaagacacgacttatcgccactggcagcagccactggtaacaggattagcagagcgaggtatgtaggcggtgctacagagttcttgaagtggtggcctaactacggctacactagaaggacagtatttggtatctgcgctctgctgaagccagttaccttcggaaaaagagttggtagctcttgatccggcaaacaaaccaccgctggtagcggtggtttttttgtttgcaagcagcagattacgcgcagaaaaaaaggatctcaagaagatcctttgatcttttctacggggtctgacgctcagtggaacgaaaactcacgttaagggattttggtcatgagattatcaaaaaggatcttcacctagatccttttggggtgggcgaagaactccagcatgagatccccgcgctggaggatcatccagccctgatagaaacagaagccactggagcacctcaaaaacaccatcatacactaaatcagtaagttggcagcatcacccgacgcactttgcgccgaataaatacctgtgacggaagatcacttcgcagaataaataaatcctggtgtccctgttgataccgggaagccctgggccaacttttggcgaaaatgagacgttgatcggcacgtaagaggttccaactttcaccataatgaaataagatcactaccgggcgtattttttgagttatcgagattttcaggagctgatagaaacagaagccactggagcacctcaaaaacaccatcatacactaaatcagtaagttggcagcatcacccgacgcactttgcgccgaataaatacctgtgacggaagatcacttcgcagaataaataaatcctggtgtccctgttgataccgggaagccctgggccaacttttggcgaaaatgagacgttgatcggcacgtaagaggttccaactttcaccataatgaaataagatcactaccgggcgtattttttgagttatcgagattttcaggagctctttggcatcgtctctcgcctgtcccctcagttcagtaatttcctgcatttgcctgtttccagtcggtagatattccacaaaacagcagggaagcagcgcttttccgctgcataaccctgcttcggggtcattatagcgattttttcggtatatccatcctttttcgcacgatatacaggattttgccaaagggttcgtgtagactttccttggtgtatccaacggcgtcagccgggcaggataggtgaagtaggcccacccgcgagcgggtgttccttcttcactgtcccttattcgcacctggcggtgctcaacgggaatcctgctctgcgaggctggccggctaccgccggcgtaacagatgagggcaagcggatggctgatgaaaccaagccaaccaggaagggcagcccacctatcaaggtgtactgccttccagacgaacgaagagcgattgaggaaaaggcggcggcggccggcatgagcctgtcggcctacctgctggccgtcggccagggctacaaaatcacgggcgtcgtggactatgagcacgtccgcgagggcgtcccggaaaacgattccgaagcccaacctttcatagaaggcggcggtggaatcgaaatctcgtgatggcaggttgggcgtcgcttggtcggtcatttcgaaaaaggttaggaatacggttagccatttgcctgcttttatatagttcatatgggattcacctttatgttgataagaaataaaagaaaatgccaataggatatcggcattttcttttgcgtttttatttgttaactgttaattgtccttgttcaaggatgctgtctttgacaacagatgttttcttgcctttgatgttcagcaggaagctcggcgcaaacgttgattgtttgtctgcgtagaatcctctgtttgtcatatagcttgtaatcacgacattgtttcctttcgcttgaggtacagcgaagtgtgagtaagtaaaggttacatcgttaggcggatcaagatccatttttaacacaaggccagttttgttcagcggcttgtatgggccagttaaagaattagaaacataaccaagcatgtaaatatcgttagacgtaatgccgtcaatcgtcatttttgatccgcgggagtcagtgaacaggtaccatttgccgttcattttaaagacgttcgcgcgttcaatttcatctgttactgtgttagatgcaatcagcggtttcatcacttttttcagtgtgtaatcatcgtttagctcaatcataccgagagcgccgtttgctaactcagccgtgcgttttttatcgctttgcagaagtttttgactttcttgacggaagaatgatgtgcttttgccatagtatgctttgttaaataaagattcttcgccttggtagccatcttcagttccagtgtttgcttcaaatactaagtatttgtggcctttatcttctacgtagtgaggatctctcagcgtatggttgtcgcctgagctgtagttgccttcatcgatgaactgctgtacattttgatacgtttttccgtcaccgtcaaagattgatttataatcctctacaccgttgatgttcaaagagctgtctgatgctgatacgttaacttgtgcagttgtcagtgtttgtttgccgtaatgtttaccggagaaatcagtgtagaataaacggatttttccgtcagatgtaaatgtggctgaacctgaccattcttgtgtttggtcttttaggatagaatcatttgcatcgaatttgtcgctgtctttaaagacgcggccagcgtttttccagctgtcaatagaagtttcgccgactttttgatagaacatgtaaatcgatgtgtcatccgcatttttaggatctccggctaatgcaaagacgatgtggtagccgtgatagtttgcgacagtgccgtcagcgttttgtaatggccagctgtcccaaacgtccaggccttttgcagaagagatatttttaattgtggacgaatcaaattcagaaacttgatatttttcatttttttgctgttcagggatttgcagcatatcatggcgtgtaatatgggaaatgccgtatgtttccttatatggcttttggttcgtttctttcgcaaacgcttgagttgcgcctcctgccagcagtgcggtagtaaaggttaatactgttgcttgttttgcaaactttttgatgttcatcgttcatgtctccttttttatgtactgtgttagcggtctgcttcttccagccctcctgtttgaagatggcaagttagttacgcacaataaaaaaagacctaaaatatgtaaggggtgacgccaaagtatacactttgccctttacacattttaggtcttgcctgctttatcagtaacaaacccgcgcgatttacttttcgacctcattctattagactctcgtttggattgcaactggtctattttcctcttttgtttgatagaaaatcataaaaggatttgcagactacgggcctaaagaactaaaaaatctatctgtttcttttcattctctgtattttttatagtttctgttgcatgggcataaagttgcctttttaatcacaattcagaaaatatcataatatctcatttcactaaataatagtgaacggcaggtatatgtgatgggttaaaaaggatcaccccagagtcccgctcagaagaactcgtcaagaaggcgatagaaggcgatgcgctgcgaatcgggagcggcgataccgtaaagcacgaggaagcggtcagcccattcgccgccaagctcttcagcaatatcacgggtagccaacgctatgtcctgatagcggtccgccacacccagccggccacagtcgatgaatccagaaaagcggccattttccaccatgatattcggcaagcaggcatcgccatgggtcacgacgagatcctcgccgtcgggcatccgcgccttgagcctggcgaacagttcggctggcgcgagcccctgatgctcttcgtccagatcatcctgatcgacaagaccggcttccatccgagtacgtgctcgctcgatgcgatgtttcgcttggtggtcgaatgggcaggtagccggatcaagcgtatgcagccgccgcattgcatcagccatgatggatactttctcggcaggagcaaggtgagatgacaggagatcctgccccggcacttcgcccaatagcagccagtcccttcccgcttcagtgacaacgtcgagacagctgcgcaaggaacgcccgtcgtggccagccacgatagccgcgctgcctcgtcttggagttcattcagggcaccggacaggtcggtcttgacaaaaagaaccgggcgcccctgcgctgacagccggaacacggcggcatcagagcagccgattgtctgttgtgcccagtcatagccgaatagcctctccacccaagcggccggagaacctgcgtgcaatccatcttgttcaatcatgcgaaacgatcctcatcctgtctcttgatcagatcttgatcccctgcgccatcagatccttggcggcaagaaagccatccagtttactttgcagggcttcccaaccttaccagagggcgccccagctggcaattccg